European Patent Application EP 4 768 501 A1, published July 1, 2026. Title: ANTI-CORONAVIRUS ANTIBODY. Applicant: CEVA SANTE ANIMALE. The sequence listing filed with the application follows.

SEQUENCE LISTING (4 sequences)

SEQ ID NO: 1 - protein, 4 aa, synthetic construct
YGMG

SEQ ID NO: 2 - protein, 17 aa, synthetic construct
GVKWSNGNTYAADSVKG

SEQ ID NO: 3 - protein, 19 aa, synthetic construct
RTGYVFGSGLYTSARWYDS

SEQ ID NO: 4 - protein, 127 aa, synthetic construct
QVQLVESGGGLVQAGGSLTLSCVVSGPGPAYGMGWFRQAPGAERVFVSGVKWSNGNTYAADSVKGRFTISRDTAKKTVYLQMNSLKPEDTAIYYCAARTGYVFGSGLYTSARWYDSWGQGTQVTVSS